European Patent Application EP 4 692 122 A1, published February 11, 2026. Title: HUMANIZED ANTIBODIES TARGETING EPHA10. Applicant: Korea University Research and Business Foundation. Application KR. The sequence listing filed with the application follows.

SEQUENCE LISTING (45 sequences)

SEQ ID NO: 1 - protein, 12 aa, synthetic construct
GFSLSTSGMGVG

SEQ ID NO: 2 - protein, 12 aa, synthetic construct
GFSLSTRGMGVG

SEQ ID NO: 3 - protein, 12 aa, synthetic construct
GFSLSTSSMGVG

SEQ ID NO: 4 - protein, 16 aa, synthetic construct
HIWWDDVKRYNPALKS

SEQ ID NO: 5 - protein, 16 aa, synthetic construct
HIRWDDVKRYNPALKS

SEQ ID NO: 6 - protein, 16 aa, synthetic construct
HIWWDDVRRYNPALKS

SEQ ID NO: 7 - protein, 11 aa, synthetic construct
ARTSFPAGVDY

SEQ ID NO: 8 - protein, 11 aa, synthetic construct
VRTSFPAGVDY

SEQ ID NO: 9 - protein, 16 aa, synthetic construct
RSSQSLQNSNGNTCLN

SEQ ID NO: 10 - protein, 16 aa, synthetic construct
RSSQSLQNSNGNTYLN

SEQ ID NO: 11 - protein, 16 aa, synthetic construct
RSSQSLQNSNGNTNLN

SEQ ID NO: 12 - protein, 16 aa, synthetic construct
RSSQSLQNSNGNTRLN

SEQ ID NO: 13 - protein, 16 aa, synthetic construct
RSSQSLQNSNGNTALN

SEQ ID NO: 14 - protein, 16 aa, synthetic construct
RSSQSLQNSNGNTWLN

SEQ ID NO: 15 - protein, 7 aa, synthetic construct
RVSNRFS

SEQ ID NO: 16 - protein, 7 aa, synthetic construct
RVSSRFS

SEQ ID NO: 17 - protein, 9 aa, synthetic construct
LQVTHVPFT

SEQ ID NO: 18 - protein, 9 aa, synthetic construct
LQGTHVPFT

SEQ ID NO: 19 - protein, 9 aa, synthetic construct
LQETHVPFT

SEQ ID NO: 20 - protein, 119 aa, synthetic construct
QVTLKESGPTLVKPTQTLTLTCTFSGFSLSTSGMGVGWIRQPPGKALEWLAHIWWDDVKRYNPALKSRLTITKDTSKNQVVLTMTNMDPVDTATYYCARTSFPAGVDYWGQGTLVTVSS

SEQ ID NO: 21 - protein, 119 aa, synthetic construct
QVTLKESGPTLVKPTQTLTLTCTFSGFSLSTRGMGVGWIRQPPGKALEWLAHIRWDDVKRYNPALKSRLTITKDTSKNQVVLTMTNMDPVDTATYYCARTSFPAGVDYWGQGTLVTVSS

SEQ ID NO: 22 - protein, 119 aa, synthetic construct
QVTLKESGPTLVKPTQTLTLTCTFSGFSLSTSGMGVGWIRKPPGKALEWLAHIWWDDVRRYNPALKSRLTITKDTSKNQVVLTMTNMDPVDTATYYCVRTSFPAGVDYWGQGTRVTVSS

SEQ ID NO: 23 - protein, 119 aa, synthetic construct
QVTLKESGPTLVKPTQTLTLTCTFSGFSLSTSSMGVGWIRQPPGKALEWLAHIRWDDVKRYNPALKSRLTITKDTSKNQVVLTMTNMDPVDTATYYCARTSFPAGVDYWGQGTLVTVSS

SEQ ID NO: 24 - protein, 119 aa, synthetic construct
RVTLKESGPTLVKPTQTLTLTCTFSGFSLSTSGMGVGWIRQPPGKALEWLAHIRWDDVKRYNPALKSRLTITKDTSKNQVVLTMTNMDPVDTATYYCARTSFPAGVDYWGQGTLVTVSS

SEQ ID NO: 25 - protein, 119 aa, synthetic construct
QVTLKESGPTLVKPTQTITLTCTFSGFSLSTSGMGVGWIRQPPGKALEWLAHIWWDDVKRYNPALKSRLTITKDTSKNQVVLTMTNMDPVDTATYYCARTSFPAGVDYWGQGTLVTVSS

SEQ ID NO: 26 - protein, 113 aa, synthetic construct
DVVMTQSPLSLPVTLGQPASISCRSSQSLQNSNGNTCLNWFQQRPGQSPRRLIYRVSNRFSGVPDRFSGSGSGTDFTLKISRVEAEDVGVYYCLQVTHVPFTFGQGTKLEIKR

SEQ ID NO: 27 - protein, 113 aa, synthetic construct
DIVMTQTPLSLSVTPGQPASISCRSSQSLQNSNGNTCLNWYLQKPGQSPQLLIYRVSNRFSGVPDRFSGSGSGTDFTLKISRVEAEDVGVYYCLQVTHVPFTFGQGTKLEIKR

SEQ ID NO: 28 - protein, 113 aa, synthetic construct
DVVMTQSPLSLPVTLGQPASISCRSSQSLQNSNGNTCLNWFQQRPGQSPRRLIYRVSSRFSGVPDRFSGSGSGTDFTLKISRVEAEDVGVYYCLQVTHVPFTFGQGTKLEIKR

SEQ ID NO: 29 - protein, 113 aa, synthetic construct
DVVMTQSPLSLPVTLGQPASISCRSSQSLQNSNGNTYLNWFQQRPGQSPRRLIYRVSNRFSGVPDRFSGSGSGTDFTLKISRVEAEDVGVYYCLQGTHVPFTFGQGTKLEIKR

SEQ ID NO: 30 - protein, 113 aa, synthetic construct
AVVMTQSPLSLPVTLGQPASISCRSSQSLQNSNGNTYLNWFQQRPGQSPRRLIYRVSNRFSGVPDRFSGSGSGTDFTLKISRVEAEDVGVYYCLQGTHVPFTFGQGTKLEIKR

SEQ ID NO: 31 - protein, 113 aa, synthetic construct
DVVMTQSPLSLPVTLGQPASISCRSSQSLQNSNGNTCLNWFQQRPGQSPRRLIYRVSNRFSGVPDRFSGSGSGTDFTLKISRVEAEDVGVYYCLQVTHVPFTFGRDTKLEIKR

SEQ ID NO: 32 - protein, 113 aa, synthetic construct
DVVMTQSPLSLPVTLGQPASISCRSSQSLQNSNGNTCLNWFQQRPGQNPRRLIYRVSNRFSGVPDRFSGSDSGTDYTLKISRVEAEDVGVYYCLQVTHVPFTFGQGTKLEIKR

SEQ ID NO: 33 - protein, 113 aa, synthetic construct
DVVMTQSPLSLPVTLGQPASISCRSSQSLQNSNGNTCLNWFQQRPGQSPRRLIYRVSNRFSGVPDRFSGSGSGTDFTLKISREEAEDVGVYYCLQVTHVPFTFGQGTKLEIKR

SEQ ID NO: 34 - protein, 113 aa, synthetic construct
DIAMTQTPMSLSVTPGQPASISCRSSQSLQNSNGNTNLNWYLQKPGQSPQLLIYRVSNRFSGVPDRFSGSGSGTDFTLKISRVEAEDVGVYYCLQVTHVPFTFGQGTKLEIKR

SEQ ID NO: 35 - protein, 113 aa, synthetic construct
DIVMTQTPLSLSVTPGQPASISCRSSQSLQNSNGNTRLNWYLQKPGQSPQLLIYRVSNRFSGVPDRFSGSGSGTDFTLKISRVEAEDVGVYYCLQETHVPFTFGQGTKLEIKR

SEQ ID NO: 36 - protein, 113 aa, synthetic construct
DVVMTQSPLSLPVTLGQPASISCRSSQSLQNSNGNTALNWFQQRPGQSPRRLIYRVSNRFSGVPDRFSGSGSGTDFTLKISRVEAEDVGVYYCLQVTHVPFTFGQGTKLEIKR

SEQ ID NO: 37 - protein, 113 aa, synthetic construct
DVVMTQSPLSLPVTLGQPASISCRSSQSLQNSNGNTNLNWFQQRPGQSPRRLIYRVSNRFSGVPDRFSGSGSGTDFTLKISRVEAEDVGVYYCLQVTHVPFTFGQGTKLEIKR

SEQ ID NO: 38 - protein, 113 aa, synthetic construct
DVVMTQSPLSLPVTLGQPASISCRSSQSLQNSNGNTRLNWFQQRPGQSPRRLIYRVSNRFSGVPDRFSGSGSGTDFTLKISRVEAEDVGVYYCLQVTHVPFTFGQGTKLEIKR

SEQ ID NO: 39 - protein, 113 aa, synthetic construct
DVVMTQSPLSLPVTLGQPASISCRSSQSLQNSNGNTWLNWFQQRPGQSPRRLIYRVSNRFSGVPDRFSGSGSGTDFTLKISRVEAEDVGVYYCLQVTHVPFTFGQGTKLEIKR

SEQ ID NO: 40 - protein, 113 aa, synthetic construct
DVVMTQSPLSLPVTLGQPASISCRSSQSLQNSNGNTYLNWFQQRPGQSPRRLIYRVSNRFSGVPDRFSGSGSGTDFTLKISRVEAEDVGVYYCLQVTHVPFTFGQGTKLEIKR

SEQ ID NO: 41 - protein, 113 aa, synthetic construct
DIVMTQTPLSLSVTPGQPASISCRSSQSLQNSNGNTALNWYLQKPGQSPQLLIYRVSNRFSGVPDRFSGSGSGTDFTLKISRVEAEDVGVYYCLQVTHVPFTFGQGTKLEIKR

SEQ ID NO: 42 - protein, 113 aa, synthetic construct
DIVMTQTPLSLSVTPGQPASISCRSSQSLQNSNGNTWLNWYLQKPGQSPQLLIYRVSNRFSGVPDRFSGSGSGTDFTLKISRVEAEDVGVYYCLQVTHVPFTFGQGTKLEIKR

SEQ ID NO: 43 - protein, 113 aa, synthetic construct
DIVMTQTPLSLSVTPGQPASISCRSSQSLQNSNGNTNLNWYLQKPGQSPQLLIYRVSNRFSGVPDRFSGSGSGTDFTLKISRVEAEDVGVYYCLQVTHVPFTFGQGTKLEIKR

SEQ ID NO: 44 - protein, 113 aa, synthetic construct
DIVMTQTPLSLSVTPGQPASISCRSSQSLQNSNGNTRLNWYLQKPGQSPQLLIYRVSNRFSGVPDRFSGSGSGTDFTLKISRVEAEDVGVYYCLQVTHVPFTFGQGTKLEIKR

SEQ ID NO: 45 - protein, 113 aa, synthetic construct
DIVMTQTPLSLSVTPGQPASISCRSSQSLQNSNGNTYLNWYLQKPGQSPQLLIYRVSNRFSGVPDRFSGSGSGTDFTLKISRVEAEDVGVYYCLQVTHVPFTFGQGTKLEIKR